European Patent Specification EP 3 496 738 B1, published August 16, 2023. Title: METHODS AND COMPOSITIONS FOR PREVENTING AND TREATING DAMAGE TO THE HEART. Applicant: MandalMed, Inc. University of California, San Francisco. Application Not Yet Assigned. The sequence listing filed with the application follows.

SEQUENCE LISTING (12 sequences)

SEQ ID NO: 1 - protein, 250 aa, Homo sapiens [sequence omitted]

SEQ ID NO: 2 - DNA, 818 bp, Artificial Sequence
  Synthetic construct
agcagccgtccggagccagccaacgagcggaaaatggcagacaatttttcgctccatgatgcgttatctgggtctggaaacccaaaccctcaaggatggcctggcgcatgggggaaccagcctgctggggcagggggctacccaggggcttcctatcctggggcctaccccgggcaggcacccccaggggcttatcctggacaggcacctccaggcgcctaccatggagcacctggagcttatcccggagcacctgcacctggagtctacccagggccacccagcggccctggggcctacccatcttctggacagccaagtgcccccggagcctaccctgccactggcccctatggcgcccctgctgggccactgattgtgccttataacctgcctttgcctgggggagtggtgcctcgcatgctcataacaattctgggcacggtgaagcccaatgcaaacagaattgctttagatttccaaagagggaatgatgttgccttccactttaacccacgcttcaatgagaacaacaggagagtcattgtttgcaatacaaagctggataataactggggaagggaagaaagacagtcggttttcccatttgaaagtgggaaaccattcaaaatacaagtactggttgaacctgaccacttcaaggttgcagtgaatgatgctcacttgttgcagtacaatcatcgggttaaaaaactcaatgaaatcagcaaactgggaatttctggtgacatagacctcaccagtgcttcatataccatgatataatctgaaaggggcagattaaaaaaaaaaacgga

SEQ ID NO: 3 - protein, 143 aa, Artificial Sequence
  Synthetic construct
GAPAGPLIVPYNLPLPGGVVPRMLITILGTVKPNANRIALDFQRGNDVAFHFNPRFNENNRRVIVCNTKLDNNWGREERQSVFPFESGKPFKIQVLVEPDHFKVAVNDAHLLQYNHRVKKLNEISKLGISGDIDITSASYTMI

SEQ ID NO: 4 - DNA, 432 bp, Artificial Sequence
  Synthetic construct
atgggcgcccctgctgggccactgattgtgccttataacctgcctttgcctgggggagtggtgcctcgcatgctcataacaattctgggcacggtgaagcccaatgcaaacagaattgctttagatttccaaagagggaatgatgttgccttccactttaacccacgcttcaatgagaacaacaggagagtcattgtttgcaatacaaagctggataataactggggaagggaagaaagacagtcggttttcccatttgaaagtgggaaaccattcaaaatacaagtactggttgaacctgaccacttcaaggttgcagtgaatgatgctcacttgttgcagtacaatcatcgggttaaaaaactcaatgaaatcagcaaactgggaatttctggtgacatagacctcaccagtgcttcatataccatgata

SEQ ID NO: 5 - DNA, 753 bp, Artificial Sequence
  Synthetic construct
atggcagataacttctcgctgcatgacgcactgtcgggctcgggtaatccgaatccgcagggctggccgggcgcttggggtaatcaaccggcaggtgccggcggttatccgggtgcttcttatccgggcgcatacccgggtcaggctccgccgggtgcatacccgggtcaagcaccgccgggtgcatatcatggtgcaccgggtgcttacccgggtgcaccggctccgggtgtgtatccgggtccgccgtcaggcccgggtgcctacccgagctctggtcagccgtcggcaccgggtgcatatccggcaacgggtccgtacggtgcaccggcaggtccgctgattgttccgtataacctgccgctgccgggcggtgtggttccgcgtatgctgattaccatcctgggcacggtcaaaccgaacgctaatcgtattgcgctggattttcaacgcggtaacgacgtggcgtttcatttcaacccgcgcttcaatgaaaacaatcgtcgcgtcatcgtgtgcaataccaaactggataacaattggggccgtgaagaacgccagagtgtttttccgttcgaatccggtaaaccgtttaaaatccaagttctggtcgaaccggatcacttcaaagtggccgttaatgacgcacatctgctgcagtataaccaccgtgtcaaaaaactgaatgaaattagtaaactgggcatttctggcgacattgacctgacctcggcgtcctacacgatgatttaa

SEQ ID NO: 6 - DNA, 432 bp, Artificial Sequence
  Synthetic construct
atgggtgcaccggcaggtccgctgattgttccgtataacctgccgctgccgggcggtgtggttccgcgtatgctgattaccatcctgggcacggtcaaaccgaacgctaatcgtattgcgctggattttcaacgcggtaacgacgtggcgtttcatttcaacccgcgcttcaatgaaaacaatcgtcgcgtcatcgtgtgcaataccaaactggataacaattggggccgtgaagaacgccagagtgtttttccgttcgaatccggtaaaccgtttaaaatccaagttctggtcgaaccggatcacttcaaagtggccgttaatgacgcacatctgctgcagtataaccaccgtgtcaaaaaactgaatgaaattagtaaactgggcatttctggcgacattgacctgacctcggcgtcctacacgatgatt

SEQ ID NO: 7 - protein, 143 aa, Artificial Sequence
  Synthetic construct
GAPAGPLIVPYNLPLPGGVVPRMLITILGTVKPNANRIALDFQRGNDVAFHFNPRFNENNRRVIVCNTKLDNNWGREERQSVFPFESGKPFKIQVLVEPEHFKVAVNDAHLLQYNHRVKKLNEISKLGISGDIDLTSASYTMI

SEQ ID NO: 8 - protein, 143 aa, Artificial Sequence
  Synthetic construct
GAPAGPLIVPYNLPLPGGVVPRMLITILGTVKPNANRIALDFQRGNDVAFHFNPRFNENNRRVIVCNTKLDNNWGREERQSVFPFESGKPFKIQVLVEPEHFKVAVNDAHLLQYNHRAKKLNEISKLGISGDIDLTSASYTMI

SEQ ID NO: 9 - DNA, 24 bp, Artificial Sequence
  Synthetic construct
gttgaacctgaacacttcaaggtt

SEQ ID NO: 10 - DNA, 27 bp, Artificial Sequence
  Synthetic construct
gacgacgacaagggcgcccctgctggg

SEQ ID NO: 11 - DNA, 30 bp, Artificial Sequence
  Synthetic construct
gaggagaagcccggtttatatcatggtata

SEQ ID NO: 12 - DNA, 24 bp, Artificial Sequence
  Synthetic construct
aatcatcgggctaaaaaactcaat